European Patent Specification EP 3 689 906 B1, published September 10, 2025. Title: IL-5 ANTIBODY, ANTIGEN BINDING FRAGMENT THEREOF, AND MEDICAL APPLICATION THEREFOR. Applicant: JIANGSU HENGRUI MEDICINE CO., LTD.; SHANGHAI HENGRUI PHARMACEUTICAL CO., LTD. The sequence listing filed with the application follows.

SEQUENCE LISTING (82 sequences)

SEQ ID NO: 1 - protein, 140 aa, Artificial sequence
  Human IL-5 amino acid sequence with his tag (rhIL-5-his)
MRMLLHLSLLALGAAYVYAIPTEIPTSALVKETLALLSTHRTLLIANETLRIPVPVHKNHQLCTEEIFQGIGTLESQTVQGGTVERLFKNLSLIKKYIDGQKKKCGEERRRVNQFLDYLQEFLGVMNTEWIIESHHHHHH

SEQ ID NO: 2 - protein, 140 aa, Artificial sequence
  Cynomolgus monkey IL-5 amino acid sequence with his tag
MRMLLHLSLLALGAAYVYAIPTEIPASALVKETLALLSTHRTLLIANETLRIPVPVHKNHQLCTEEIFQGIGTLESQTVQGGTVERLFKNLSLIKKYIGGQKKKCGEERRRVNQFLDYLQEFLGVMNTEWIIESHHHHHH

SEQ ID NO: 3 - protein, 119 aa, Artificial sequence
  Mouse IL-5 amino acid sequence with his tag
MEIPMSTVVKETLTQLSAHRALLTSNETMRLPVPTHKNHQLCIGEIFQGLDILKNQTVRGGTVEMLFQNLSLIKKYIDRQKEKCGEERRRTRQFLDYLQEFLGVMSTEWAMEGHHHHHH

SEQ ID NO: 4 - protein, 119 aa, Artificial sequence
  Rat IL-5 amino acid sequence with his tag
MEIPMSTVVKETLIQLSTHRALLTSNETMRLPVPTHKNHQLCIGEIFQGLDILKNQTVRGGTVEILFQNLSLIKKYIDGQKEKCGEERRKTRHFLDYLQEFLGVMSTEWAMEVHHHHHH

SEQ ID NO: 5 - protein, 560 aa, Artificial sequence
  human IL-5 alpha fused to human Fc fragment
DLLPDEKISLLPPVNFTIKVTGLAQVLLQWKPNPDQEQRNVNLEYQVKINAPKEDDYETRITESKCVTILHKGFSASVRTILQNDHSLLASSWASAELHAPPGSPGTSIVNLTCTTNTTEDNYSRLRSYQVSLHCTWLVGTDAPEDTQYFLYYRYGSWTEECQEYSKDTLGRNIACWFPRTFILSKGRDWLAVLVNGSSKHSAIRPFDQLFALHAIDQINPPLNVTAEIEGTRLSIQWEKPVSAFPIHCFDYEVKIHNTRNGYLQIEKLMTNAFISIIDDLSKYDVQVRAAVSSMCREAGLWSEWSQPIYVGNDEHKPLREWIEGRMDEPKSCDKTHTCPPCPAPELLGGPSVFLFPPKPKDTLMISRTPEVTCVVVDVSHEDPEVKFNWYVDGVEVHNAKTKPREEQYNSTYRVVSVLTVLHQDWLNGKEYKCKVSNKALPAPIEKTISKAKGQPREPQVYTLPPSRDELTKNQVSLTCLVKGFYPSDIAVEWESNGQPENNYKTTPPVLDSDGSFFLYSKLTVDKSRWQQGNVFSCSVMHEALHNHYTQKSLSLSPGK

SEQ ID NO: 6 - protein, 118 aa, Artificial sequence
  mAb1705 murine heavy chain variable region sequence
EVQLVESGGGLVQPGRSLKLSCTASGFTFSHYYMAWVRQAPKKGLEWVTSISYEGDITYYGDSVKGRFTISRDNAKSTLYLQMNSLRSEDTATYYCASQTLRESFDYWGQGVMVTVSS

SEQ ID NO: 7 - protein, 107 aa, Artificial sequence
  mAb1705 murine light chain variable region sequence
DIQMTQSPSSMSVSLGDRVTITCRASQDIANYLSWYQQKIARSPKLVIYGTSNLEVGVPSRFSGSRSGSDYSLTINTLESEDTGIYFCLQDKEFPRTFGGGTRLELK

SEQ ID NO: 8 - protein, 118 aa, Artificial sequence
  mAb1706 murine heavy chain variable region sequence
EVQLVESGGGLVQPGRSLKLSCAASGFTFSHYYMAWVRQAPKKGLEWVTSINYEGNSAYYGDSVKGRFTISRDNAKSTLYLQMDSLRSEDTATYYCATETLRESLDYWGQGVMVTVSS

SEQ ID NO: 9 - protein, 107 aa, Artificial sequence
  mAb1706 murine light chain variable region sequence
DIQMTQSPSSMSVSLGDRVTITCRASQDIGNYLSWYQQKLGKSPKLMIHSASNLEVGVPSRFSGSRSGSDYSLTINTLESEDPGIYFCLQHKQFPRTFGGGTKLELK

SEQ ID NO: 10 - protein, 119 aa, Artificial sequence
  mAb1780 murine heavy chain variable region sequence
QVKLLQSGAALVKPGDSVKMSCKASDYTFTEYLIHWVKQSQGRSLEWIGYINPYSGGTVYNEKFKSKATLTVDKFSSTAYMEFRRLTFEDSAIYYCARDGGYSDPLDYWGQGVMVTVSS

SEQ ID NO: 11 - protein, 106 aa, Artificial sequence
  mAb1780 murine light chain variable region sequence
DTVLTQSPALAVSPGERVSISCRASEGLTSYMHWYQQKPGQQPKLLIYKASNLASGVPARFSGSGSGTDFTLTIDPVEADDAATYFCQQNWNDPWTFGGGTKLELK

SEQ ID NO: 12 - protein, 116 aa, Artificial sequence
  mAb1773 murine heavy chain variable region sequence
EVQLQQSLAELVRPGASVTLSCTASGFNIKNTYIHWVKQRPEQGLEWIGRIDPANGDTKHGPKFQGKATITADTSSNTAYLQFSSLTSEDTAIYYCFRYGIYPDHWGQGTPLTVSS

SEQ ID NO: 13 - protein, 106 aa, Artificial sequence
  mAb1773 murine light chain variable region sequence
QIVLTQSPALMSASPGEKVTMTCSASSSVNYIYWYQQKPRSSPKPWIYLTATLASGVPARFSGSGSGTSFSLTISRMEAEDAATYYCQQWNSYPYTFGGGTKLEIE

SEQ ID NO: 14 - protein, 120 aa, Artificial sequence
  mAb1779 murine heavy chain variable region sequence
QVKLLQSGAALVKPGDSVKMSCKASGYTFTDYIIHWVKQSHGKSLEWIGYFNPNSGGSNYNENFKRKATLTADKSSSTAYLEFSRVTSEDSAIYYCGRRIAWDHWYFDFWGPGTMVTVSS

SEQ ID NO: 15 - protein, 107 aa, Artificial sequence
  mAb1779 murine light chain variable region sequence
DIQMTQSPASLSASLGETVSIECLASEGISNDVAWYQQKSGRSPQLLVYAASRLQDGVPSRFSGSGSGTRYFFKISGMQPEDEADYFCQQGYKTPLTFGSGTKLEIK

SEQ ID NO: 16 - protein, 5 aa, Artificial sequence
  mAb1705 HCDR1
HYYMA

SEQ ID NO: 17 - protein, 17 aa, Artificial sequence
  mAb1705 HCDR2
SISYEGDITYYGDSVKG

SEQ ID NO: 18 - protein, 9 aa, Artificial sequence
  mAb1705 HCDR3
QTLRESFDY

SEQ ID NO: 19 - protein, 11 aa, Artificial sequence
  mAb1705 LCDR1
RASQDIANYLS

SEQ ID NO: 20 - protein, 7 aa, Artificial sequence
  mAb1705 LCDR2
GTSNLEV

SEQ ID NO: 21 - protein, 9 aa, Artificial sequence
  mAb1705 LCDR3
LQDKEFPRT

SEQ ID NO: 22 - protein, 5 aa, Artificial sequence
  mAb1706 HCDR1
HYYMA

SEQ ID NO: 23 - protein, 17 aa, Artificial sequence
  mAb1706 HCDR2
SINYEGNSAYYGDSVKG

SEQ ID NO: 24 - protein, 9 aa, Artificial sequence
  mAb1706 HCDR3
ETLRESLDY

SEQ ID NO: 25 - protein, 11 aa, Artificial sequence
  mAb1706 LCDR1
RASQDIGNYLS

SEQ ID NO: 26 - protein, 7 aa, Artificial sequence
  mAb1706 LCDR2
SASNLEV

SEQ ID NO: 27 - protein, 9 aa, Artificial sequence
  mAb1706 LCDR3
LQHKQFPRT

SEQ ID NO: 28 - protein, 5 aa, Artificial sequence
  mAb1780 HCDR1
EYLIH

SEQ ID NO: 29 - protein, 17 aa, Artificial sequence
  mAb1780 HCDR2
YINPYSGGTVYNEKFKS

SEQ ID NO: 30 - protein, 10 aa, Artificial sequence
  mAb1780 HCDR3
DGGYSDPLDY

SEQ ID NO: 31 - protein, 11 aa, Artificial sequence
  mAb1780 LCDR1
RASEGLTSYMH

SEQ ID NO: 32 - protein, 7 aa, Artificial sequence
  mAb1780 LCDR2
KASNLAS

SEQ ID NO: 33 - protein, 9 aa, Artificial sequence
  mAb1780 LCDR3
QQNWNDPWT

SEQ ID NO: 34 - protein, 5 aa, Artificial sequence
  mAb1773 HCDR1
NTYIH

SEQ ID NO: 35 - protein, 17 aa, Artificial sequence
  mAb1773 HCDR2
RIDPANGDTKHGPKFQG

SEQ ID NO: 36 - protein, 7 aa, Artificial sequence
  mAb1773 HCDR3
YGIYPDH

SEQ ID NO: 37 - protein, 10 aa, Artificial sequence
  mAb1773 LCDR1
SASSSVNYIY

SEQ ID NO: 38 - protein, 7 aa, Artificial sequence
  mAb1773 LCDR2
LTATLAS

SEQ ID NO: 39 - protein, 9 aa, Artificial sequence
  mAb1773 LCDR3
QQWNSYPYT

SEQ ID NO: 40 - protein, 5 aa, Artificial sequence
  mAb1779 HCDR1
DYIIH

SEQ ID NO: 41 - protein, 17 aa, Artificial sequence
  mAb1779 HCDR2
YFNPNSGGSNYNENFKR

SEQ ID NO: 42 - protein, 11 aa, Artificial sequence
  mAb1779 HCDR3
RIAWDHWYFDF

SEQ ID NO: 43 - protein, 11 aa, Artificial sequence
  mAb1779 LCDR1
LASEGISNDVA

SEQ ID NO: 44 - protein, 7 aa, Artificial sequence
  mAb1779 LCDR2
AASRLQD

SEQ ID NO: 45 - protein, 9 aa, Artificial sequence
  mAb1779 LCDR3
QQGYKTPLT

SEQ ID NO: 46 - protein, 107 aa, Artificial sequence
  h1705_VL.1
DIQMTQSPSSVSASVGDRVTITCRASQDIANYLSWYQQKPGKAPKLLIYGTSNLEVGVPSRFSGSGSGTDFTLTISSLQPEDFATYYCLQDKEFPRTFGGGTKVEIK

SEQ ID NO: 47 - protein, 107 aa, Artificial sequence
  h1705_VL.1A
DIQMTQSPSSVSASVGDRVTITCRASQDIANYLSWYQQKPGKSPKLLIYGTSNLEVGVPSRFSGSRSGTDFTLTISSLQPEDFATYYCLQDKEFPRTFGGGTKVEIK

SEQ ID NO: 48 - protein, 107 aa, Artificial sequence
  h1705_VL.1B
DIQMTQSPSSVSASVGDRVTITCRASQDIANYLSWYQQKPGKSPKLVIYGTSNLEVGVPSRFSGSRSGSDYTLTISSLQPEDFATYFCLQDKEFPRTFGGGTKVEIK

SEQ ID NO: 49 - protein, 118 aa, Artificial sequence
  h1705_VH.1
EVQLVESGGGLVQPGGSLRLSCAASGFTFSHYYMAWVRQAPGKGLEWVSSISYEGDITYYGDSVKGRFTISRDNSKNTLYLQMNSLRAEDTAVYYCAKQTLRESFDYWGQGTLVTVSS

SEQ ID NO: 50 - protein, 118 aa, Artificial sequence
  h1705_VH.1A
EVQLVESGGGLVQPGGSLRLSCAASGFTFSHYYMAWVRQAPGKGLEWVSSISYEGDITYYGDSVKGRFTISRDNSKNTLYLQMNSLRAEDTAVYYCASQTLRESFDYWGQGTLVTVSS

SEQ ID NO: 51 - protein, 118 aa, Artificial sequence
  h1705_VH.1B
EVQLVESGGGLVQPGGSLRLSCAASGFTFSHYYMAWVRQAPGKGLEWVTSISYEGDITYYGDSVKGRFTISRDNSKNTLYLQMNSLRAEDTATYYCASQTLRESFDYWGQGTLVTVSS

SEQ ID NO: 52 - protein, 330 aa, Artificial sequence
  Heavy chain IgG1 constant region
ASTKGPSVFPLAPSSKSTSGGTAALGCLVKDYFPEPVTVSWNSGALTSGVHTFPAVLQSSGLYSLSSVVTVPSSSLGTQTYICNVNHKPSNTKVDKKVEPKSCDKTHTCPPCPAPELLGGPSVFLFPPKPKDTLYITREPEVTCVVVDVSHEDPEVKFNWYVDGVEVHNAKTKPREEQYNSTYRVVSVLTVLHQDWLNGKEYKCKVSNKALPAPIEKTISKAKGQPREPQVYTLPPSRDELTKNQVSLTCLVKGFYPSDIAVEWESNGQPENNYKTTPPVLDSDGSFFLYSKLTVDKSRWQQGNVFSCSVMHEALHNHYTQKSLSLSPGK

SEQ ID NO: 53 - protein, 107 aa, Artificial sequence [sequence omitted]

SEQ ID NO: 54 - protein, 107 aa, Artificial sequence
  h1706_VL.1
DIQMTQSPSSVSASVGDRVTITCRASQDIGNYLSWYQQKPGKAPKLLIYSASNLEVGVPSRFSGSGSGTDFTLTISSLQPEDFATYYCLQHKQFPRTFGGGTKVEIK

SEQ ID NO: 55 - protein, 107 aa, Artificial sequence
  h1706_VL.1A
DIQMTQSPSSVSASVGDRVTITCRASQDIGNYLSWYQQKPGKSPKLLIYSASNLEVGVPSRFSGSGSGTDFTLTISSLQPEDFATYYCLQHKQFPRTFGGGTKVEIK

SEQ ID NO: 56 - protein, 107 aa, Artificial sequence
  h1706_VL.1B
DIQMTQSPSSVSASVGDRVTITCRASQDIGNYLSWYQQKPGKSPKLMIYSASNLEVGVPSRFSGSGSGTDYTLTISSLQPEDFATYFCLQHKQFPRTFGGGTKVEIK

SEQ ID NO: 57 - protein, 118 aa, Artificial sequence
  h1706_VH.1
EVQLVESGGGLVQPGGSLRLSCAASGFTFSHYYMAWVRQAPGKGLEWVSSINYEGNSAYYGDSVKGRFTISRDNSKNTLYLQMNSLRAEDTAVYYCAKETLRESLDYWGQGTMVTVSS

SEQ ID NO: 58 - protein, 118 aa, Artificial sequence
  h1706_VH.1A
EVQLVESGGGLVQPGGSLRLSCAASGFTFSHYYMAWVRQAPGKGLEWVSSINYEGNSAYYGDSVKGRFTISRDNSKNTLYLQMNSLRAEDTAVYYCATETLRESLDYWGQGTMVTVSS

SEQ ID NO: 59 - protein, 118 aa, Artificial sequence
  h1706_VH.1B
EVQLVESGGGLVQPGGSLRLSCAASGFTFSHYYMAWVRQAPGKGLEWVTSINYEGNSAYYGDSVKGRFTISRDNSKNTLYLQMNSLRAEDTATYYCATETLRESLDYWGQGTMVTVSS

SEQ ID NO: 60 - protein, 107 aa, Artificial sequence
  h1780_VL.1
EIVLTQSPATLSLSPGERATLSCRASEGLTSYMHWYQQKPGQAPRLLIYKASNLASGIPARFSGSGSGTDFTLTISSLEPEDFAVYYCQQNWNDPWTFGGGTKVEIK

SEQ ID NO: 61 - protein, 107 aa, Artificial sequence
  h1780_VL.1A
DTVLTQSPATLSLSPGERATLSCRASEGLTSYMHWYQQKPGQAPRLLIYKASNLASGIPARFSGSGSGTDFTLTISSLEPEDFAVYYCQQNWNDPWTFGGGTKVEIK

SEQ ID NO: 62 - protein, 107 aa, Artificial sequence
  h1780_VL.1B
DTVLTQSPATLSLSPGERATLSCRASEGLTSYMHWYQQKPGQAPRLLIYKASNLASGVPARFSGSGSGTDFTLTISSLEPEDFATYFCQQNWNDPWTFGGGTKVEIK

SEQ ID NO: 63 - protein, 119 aa, Artificial sequence
  h1780_VH.1
EVQLVQSGAEVKKPGASVKVSCKASGYTFTEYLIHWVRQAPGQGLEWMGYINPYSGGTVYNEKFKSRVTMTRDTSISTAYMELSRLRSDDTAVYYCARDGGYSDPLDYWGQGTMVTVSS

SEQ ID NO: 64 - protein, 119 aa, Artificial sequence
  h1780_VH.1A
EVQLVQSGAEVKKPGASVKVSCKASGYTFTEYLIHWVRQAPGQGLEWMGYINPYSGGTVYNEKFKSRVTLTVDKSISTAYMELSRLRSDDTAVYYCARDGGYSDPLDYWGQGTMVTVSS

SEQ ID NO: 65 - protein, 119 aa, Artificial sequence
  h1780_VH.1B
EVQLVQSGAEVKKPGASVKVSCKASGYTFTEYLIHWVRQAPGQGLEWIGYINPYSGGTVYNEKFKSRATLTVDKSISTAYMEFSRLRSDDTAVYYCARDGGYSDPLDYWGQGTMVTVSS

SEQ ID NO: 66 - protein, 119 aa, Artificial sequence
  h1780_VH.1C
EVQLVQSGAEVKKPGASVKVSCKASGYTFTEYLIHWVKQAPGQGLEWIGYINPYSGGTVYNEKFKSKATLTVDKSISTAYMEFSRLRSDDTAVYYCARDGGYSDPLDYWGQGTMVTVSS

SEQ ID NO: 67 - protein, 106 aa, Artificial sequence
  h1773_VL.1
DIQMTQSPSSLSASVGDRVTITCSASSSVNYIYWYQQKPGKAPKLLIYLTATLASGVPSRFSGSGSGTDFTLTISSLQPEDFATYYCQQWNSYPYTFGGGTKVEIK

SEQ ID NO: 68 - protein, 106 aa, Artificial sequence
  h1773_VL.1A
DIQLTQSPSSLSASVGDRVTITCSASSSVNYIYWYQQKPGKSPKPWIYLTATLASGVPSRFSGSGSGTDFTLTISSLQPEDFATYYCQQWNSYPYTFGGGTKVEIK

SEQ ID NO: 69 - protein, 116 aa, Artificial sequence
  h1773_VH.1
EVQLVESGGGLVQPGGSLKLSCAASGFTFSNTYIHWVRQASGKGLEWVGRIDPAVGDTKHGPKFQGRFTISRDDSKNTAYLQMNSLKTEDTAVYYCTRYGIYPDHWGQGTLVTVSS

SEQ ID NO: 70 - protein, 116 aa, Artificial sequence
  h1773_VH.1A
EVQLVESGGGLVQPGGSLKLSCAASGFTISNTYIHWVRQASGKGLEWVGRIDPAVGDTKHGPKFQGRFTISADDSKNTAYLQMNSLKTEDTAVYYCFRYGIYPDHWGQGTLVTVSS

SEQ ID NO: 71 - protein, 116 aa, Artificial sequence
  h1773_VH.1B
EVQLVESGGGLVQPGGSLKLSCAASGFTISNTYIHWVKQASGKGLEWIGRIDPAVGDTKHGPKFQGRFTISADDSKNTAYLQMNSLKTEDTAVYYCFRYGIYPDHWGQGTLVTVSS

SEQ ID NO: 72 - protein, 107 aa, Artificial sequence
  h1779_VL.1
DIQMTQSPSSLSASVGDRVTITCLASEGISNDVAWYQQKPGKAPKLLIYAASRLQDGVPSRFSGSGSGTDFTFTISSLQPEDIATYYCQQGYKTPLTFGQGTKLEIK

SEQ ID NO: 73 - protein, 107 aa, Artificial sequence
  h1779_VL.1A
DIQMTQSPSSLSASVGDRVTITCLASEGISNDVAWYQQKPGKSPKLLIYAASRLQDGVPSRFSGSGSGTDFTFTISSLQPEDIATYYCQQGYKTPLTFGQGTKLEIK

SEQ ID NO: 74 - protein, 107 aa, Artificial sequence
  h1779_VL.1B
DIQMTQSPSSLSASVGDRVTITCLASEGISNDVAWYQQKPGKSPKLLVYAASRLQDGVPSRFSGSGSGTDYTFTISSLQPEDIATYYCQQGYKTPLTFGQGTKLEIK

SEQ ID NO: 75 - protein, 120 aa, Artificial sequence
  h1779_VH.1
EVQLVQSGAEVKKPGASVKVSCKASGYTFTDYIIHWVRQAPGQGLEWMGYFNPNSGGSNYNENFKRRVTMTRDTSISTAYMELSRLRSEDTAVYYCARRIAWDHWYFDFWGQGTMVTVSS

SEQ ID NO: 76 - protein, 120 aa, Artificial sequence
  h1779_VH.1A
EVQLVQSGAEVKKPGASVKVSCKASGYTFTDYIIHWVRQAPGQGLEWMGYFNPNSGGSNYNENFKRRVTMTADKSISTAYMELSRLRSEDTAVYYCARRIAWDHWYFDFWGQGTMVTVSS

SEQ ID NO: 77 - protein, 120 aa, Artificial sequence
  h1779_VH.1B
EVQLVQSGAEVKKPGASVKVSCKASGYTFTDYIIHWVRQAPGQGLEWIGYFNPNSGGSNYNENFKRRATMTADKSISTAYMELSRLRSEDTAVYYCARRIAWDHWYFDFWGQGTMVTVSS

SEQ ID NO: 78 - protein, 120 aa, Artificial sequence
  h1779_VH.1C
EVQLVQSGAEVKKPGASVKVSCKASGYTFTDYIIHWVRQAPGQGLEWIGYFNPNSGGSNYNENFKRRATMTADKSISTAYLEFSRLRSEDTAVYYCARRIAWDHWYFDFWGQGTMVTVSS

SEQ ID NO: 79 - protein, 120 aa, Artificial sequence
  h1779_VH.1D
EVQLVQSGAEVKKPGASVKVSCKASGYTFTDYIIHWVKQAPGQGLEWIGYFNPNSGGSNYNENFKRKATMTADKSISTAYLEFSRLRSEDTAVYYCARRIAWDHWYFDFWGQGTMVTVSS

SEQ ID NO: 80 - protein, 443 aa, Artificial sequence
  Heavy chain sequence of Hu39D10
EVQLVESGGGLVQPGGSLRLSCAVSGLSLTSNSVNWIRQAPGKGLEWVGLIWSNGDTDYNSAIKSRFTISRDTSKSTVYLQMNSLRAEDTAVYYCAREYYGYFDYWGQGTLVTVSSASTKGPSVFPLAPCSRSTSESTAALGCLVKDYFPEPVTVSWNSGALTSGVHTFPAVLQSSGLYSLSSVVTVPSSSLGTKTYTCNVDHKPSNTKVDKRVESKYGPPCPPCPAPEFLGGPSVFLFPPKPKDTLMISRTPEVTCVVVDVSQEDPEVQFNWYVDGVEVHNAKTKPREEQFNSTYRVVSVLTVLHQDWLNGKEYKCKVSNKGLPSSIEKTISKAKGQPREPQVYTLPPSQEEMTKNQVSLTCLVKGFYPSDIAVEWESNGQPENNYKTTPPVLDSDGSFFLYSRLTVDKSRWQEGNVFSCSVMHEALHNHYTQKSLSLSLGK

SEQ ID NO: 81 - protein, 214 aa, Artificial sequence
  Light chain sequence of Hu39D10
DIQMTQSPSSLSASVGDRVTITCLASEGISSYLAWYQQKPGKAPKLLIYGANSLQTGVPSRFSGSGSATDYTLTISSLQPEDFATYYCQQSYKFPNTFGQGTKVEVKRTVAAPSVFIFPPSDEQLKSGTASVVCLLNNFYPREAKVQWKVDNALQSGNSQESVTEQDSKDSTYSLSSTLTLSKADYEKHKVYACEVTHQGLSSPVTKSFNRGEC

SEQ ID NO: 82 - protein, 17 aa, Artificial sequence
  h1773 antibody body heavy chain HCDR2 variant
RIDPAVGDTKHGPKFQG